European Patent Application EP 4 477 236 A1, published December 18, 2024. Title: COMBINATION THERAPY FOR TREATING A TUMOR USING ADC COMPRISING ANTI-CD71 ANTIBODIES AND BH3 MIMETICS. Applicant: INATHERYS. The sequence listing filed with the application follows.

SEQUENCE LISTING (20 sequences)

SEQ ID NO: 1 - protein, 7 aa, Homo sapiens
GYTFTNQ

SEQ ID NO: 2 - protein, 6 aa, Homo sapiens
NTYTGE

SEQ ID NO: 3 - protein, 8 aa, Homo sapiens
EGWDSMDY

SEQ ID NO: 4 - protein, 10 aa, Homo sapiens
SASSSVNYMH

SEQ ID NO: 5 - protein, 7 aa, Homo sapiens
STSNRAT

SEQ ID NO: 6 - protein, 9 aa, Homo sapiens
QQRSSYPLT

SEQ ID NO: 7 - protein, 7 aa, Homo sapiens
STSNLAS

SEQ ID NO: 8 - protein, 7 aa, Homo sapiens
STSNRAS

SEQ ID NO: 9 - protein, 117 aa, Homo sapiens
QIQLVQSGPELKKPGETVKISCKASGYTFTNQGMNWVKQAPGKGLKWMGWINTYTGEPINADDFKGRFAISLETSASTAYLQINNLKNEDMATYFCVREGWDSMDYWGQGTSVTVSS

SEQ ID NO: 10 - protein, 107 aa, Homo sapiens
QIVLTQSPAIMSASPGEKVTITCSASSSVNYMHWFQQKPGTSPKLWIYSTSNLASGVPARFSGSGSGTSYSLTISRMEAEDAATYYCQQRSSYPLTFGAGTKLELKR

SEQ ID NO: 11 - protein, 117 aa, Homo sapiens
QVQLVQSGPELKKPGASVKVSCKASGYTFTNQGMNWVKQAPGKGLKWMGWINTYTGEPINADDFKGRFVISLDTSASTAYLQISSLKAEDTAVYFCVREGWDSMDYWGQGTSVTVSS

SEQ ID NO: 12 - protein, 136 aa, Homo sapiens
MEWSWVFLFFLSVTTGVHSQVQLVQSGPELKKPGASVKVSCKASGYTFTNQGMNWVKQAPGKGLKWMGWINTYTGEPINADDFKGRFVISLETSASTAYLQISNLKNEDTAVYFCVREGWDSMDYWGQGTSVTVSS

SEQ ID NO: 13 - protein, 107 aa, Homo sapiens
QIVLTQSPATLSVSPGERATLSCSASSSVNYMHWFQQKPGQSPRLLIYSTSNRATGIPARFSGSGSGTSYTLTISSLEPEDFAVYYCQQRSSYPLTFGQGTKLEIKR

SEQ ID NO: 14 - protein, 107 aa, Homo sapiens
QIVLTQSPATLSLSPGERATLSCSASSSVNYMHWFQQKPGQSPRLLIYSTSNRASGVPARFSGSGSGTSYTLTISRLEPEDFAVYYCQQRSSYPLTFGQGTKLEIKR

SEQ ID NO: 15 - protein, 107 aa, Homo sapiens
QIVLTQSPATLSLSPGERATLSCSASSSVNYMHWFQQKPGQSPRLLIYSTSNLASGVPARFSGSGSGTSYTLTISRLEPEDAAVYYCQQRSSYPLTFGAGTKLELKR

SEQ ID NO: 16 - protein, 760 aa, Homo sapiens
MMDQARSAFSNLFGGEPLSYTRFSLARQVDGDNSHVEMKLAVDEEENADNNTKANVTKPKRCSGSICYGTIAVIVFFLIGFMIGYLGYCKGVEPKTECERLAGTESPVREEPGEDFPAARRLYWDDLKRKLSEKLDSTDFTGTIKLLNENSYVPREAGSQKDENLALYVENQFREFKLSKVWRDQHFVKIQVKDSAQNSVIIVDKNGRLVYLVENPGGYVAYSKAATVTGKLVHANFGTKKDFEDLYTPVNGSIVIVRAGKITFAEKVANAESLNAIGVLIYMDQTKFPIVNAELSFFGHAHLGTGDPYTPGFPSFNHTQFPPSRSSGLPNIPVQTISRAAAEKLFGNMEGDCPSDWKTDSTCRMVTSESKNVKLTVSNVLKEIKILNIFGVIKGFVEPDHYVVVGAQRDAWGPGAAKSGVGTALLLKLAQMFSDMVLKDGFQPSRSIIFASWSAGDFGSVGATEWLEGYLSSLHLKAFTYINLDKAVLGTSNFKVSASPLLYTLIEKTMQNVKHPVTGQFLYQDSNWASKVEKLTLDNAAFPFLAYSGIPAVSFCFCEDTDYPYLGTTMDTYKELIERIPELNKVARAAAEVAGQFVIKLTHDVELNLDYERYNSQLLSFVRDLNQYRADIKEMGLSLQWLYSARGDFFRATSRLTTDFGNAEKTDRFVMKKLNDRVMRVEYHFLSPYVSPKESPFRHVFWGSGSHTLPALLENLKLRKQNNGAFNETLFRNQLALATWTIQGAANALSGDVWDIDNEF

SEQ ID NO: 17 - protein, 233 aa, Homo sapiens
MSVPTQVLGLLLLWLTDARCQIVLTQSPATLSVSPGERATLSCSASSSVNYMHWFQQKPGQSPRLLIYSTSNRATGIPARFSGSGSGTSYTLTISSLEPEDFAVYYCQQRSSYPLTFGQGTKLEIKRTVAAPSVFIFPPSDEQLKSGTASVVCLLNNFYPREAKVQWKVDNALQSGNSQESVTEQDSKDSTYSLSSTLTLSKADYEKHKVYACEVTHQGLSSPVTKSFNRGEC

SEQ ID NO: 18 - protein, 462 aa, Homo sapiens
MEWSWVFLFFLSVTTGVHSQVQLVQSGPELKKPGASVKVSCKASGYTFTNQGMNWVKQAPGKGLKWMGWINTYTGEPINADDFKGRFVISLDTSASTAYLQISSLKAEDTAVYFCVREGWDSMDYWGQGTSVTVSSASTKGPSVFPLAPCSRSTSESTAALGCLVKDYFPEPVTVSWNSGALTSGVHTFPAVLQSSGLYSLSSVVTVPSSSLGTKTYTCNVDHKPSNTKVDKRVESKYGPPCPPCPAPEFLGGPSVFLFPPKPKDTLMISRTPEVTCVVVDVSQEDPEVQFNWYVDGVEVHNAKTKPREEQFNSTYRVVSVLTVLHQDWLNGKEYKCKVSNKGLPSSIEKTISKAKGQPREPQVYTLPPSQEEMTKNQVSLTCLVKGFYPSDIAVEWESNGQPENNYKTTPPVLDSDGSFFLYSRLTVDKSRWQEGNVFSCSVMHEALHNHYTQKSLSLSLG

SEQ ID NO: 19 - DNA, 724 bp, Homo sapiens
  source 1..724: mol_type = genomic DNA
aagcttgccgccaccatgtccgtgcctacccaggtgctgggactgctgctgctgtggctgaccgatgccaggtgccagatcgtgctgacccagtctcctgccaccctgtctgtgtctcccggcgagagagctaccctgtcctgctccgcctcctcctccgtgaactacatgcactggttccagcagaagcccggccagtcccccagactgctgatctactccacctccaaccgggccaccggcatccctgccagattttccggctctggctccggcacctcctataccctgaccatctccagcctggaacccgaggacttcgccgtgtactactgccagcagcggtcctcctaccccctgacctttggccagggcaccaagctggaaatcaagcgtacggtggccgctcccagcgtgttcatcttccccccaagcgacgagcagctgaagagcggcaccgccagcgtggtgtgtctgctgaacaacttctaccccagggaggccaaggtgcagtggaaggtggacaacgccctgcagagcggcaacagccaggagagcgtcaccgagcaggacagcaaggactccacctacagcctgagcagcaccctgaccctgagcaaggccgactacgagaagcacaaggtgtacgcctgtgaggtgacccaccagggcctgtccagccccgtgaccaagagcttcaacaggggcgagtgctgatgaattc

SEQ ID NO: 20 - DNA, 1411 bp, Homo sapiens
  source 1..1411: mol_type = genomic DNA
aagcttgccgccaccatggaatggtcctgggtgttcctgttcttcctgtccgtgaccaccggcgtgcactcccaggtgcagctggtgcagtctggccccgagctgaagaaacctggcgcctccgtgaaggtgtcctgcaaggcttccggctacacctttacaaaccagggcatgaactgggtcaagcaggcccctggcaagggcctgaagtggatgggctggatcaacacctacaccggcgagcccatcaacgccgacgacttcaagggcagattcgtgatctccctggacacctccgcctccaccgcctacctgcagatcagctctctgaaggccgaggataccgccgtgtacttctgcgtgcgggaaggctgggactccatggactattggggccagggcacctccgtgaccgtgtctagcgcttctacaaagggcccaagcgtgttccccctggccccctgctccagaagcaccagcgagagcacagccgccctgggctgcctggtgaaggactacttccccgagcccgtgaccgtgtcctggaacagcggagccctgaccagcggcgtgcacaccttccccgccgtgctgcagagcagcggcctgtacagcctgagcagcgtggtgaccgtgcccagcagcagcctgggcaccaagacctacacctgtaacgtggaccacaagcccagcaacaccaaggtggacaagagggtggagagcaagtacggcccaccctgccccccctgcccagcccccgagttcctgggcggacccagcgtgttcctgttcccccccaagcccaaggacaccctgatgatcagcagaacccccgaggtgacctgtgtggtggtggacgtgtcccaggaggaccccgaggtccagttcaactggtacgtggacggcgtggaggtgcacaacgccaagaccaagcccagagaggagcagtttaacagcacctaccgggtggtgtccgtgctgaccgtgctgcaccaggactggctgaacggcaaagagtacaagtgtaaggtctccaacaagggcctgccaagcagcatcgaaaagaccatcagcaaggccaagggccagcctagagagccccaggtctacaccctgccacccagccaagaggagatgaccaagaaccaggtgtccctgacctgtctggtgaagggcttctacccaagcgacatcgccgtggagtgggagagcaacggccagcccgagaacaactacaagaccacccccccagtgctggacagcgacggcagcttcttcctgtacagcaggctgaccgtggacaagtccagatggcaggagggcaacgtctttagctgctccgtgatgcacgaggccctgcacaaccactacacccagaagagcctgagcctgtccctgggctgatgaattc